European Patent Application EP 4 130 255 A1, published February 8, 2023. Title: Recombinant vector for transformation to improve glutamine production capacity and recombinant strain which introduced the same. Applicant: Daesang Corporation. The sequence listing filed with the application follows.

SEQUENCE LISTING (22 sequences)

SEQ ID NO: 1 - protein, 477 aa, Artificial Sequence
  KFCC10694 GS
VAFNTPEEIVKFIKDENVEFVDVRFTDVPGTEQHFSIPAALFDEEAIEEGLAFDGSSIRGFTTIDESDMNLLPDLGTATIDPFRKAKTLNIKFFVHDPFTREAFSRDPRNVARKAEQYLASTGIADTCNFGAEAEFYLFDSVRYSTDINSSFYHVDTNEGWWNRGRETNLDGTPNLGAKNRVKGGYFPVAPYDQTVEIRDDMVNYLSNAGFQLERFHHEVGGGQQEINYRFNTMLHAADDIQTFKYIIKNTAHLHGKTATFMPKPLAGDNGSGMHAHQSLWKDGKPLFHDESGYAGLSDIARYYIGGILHHAGAVLAFTNPTLNSYHRLVPGFEAPINLVYSQRNRSAAVRIPITGSNPKAKRIEFRAPDPSGNPYFGFAAMMMAGLDGIKNRIEPHAPVDKDLYELPPEEAASIPQAPTSLEASLKALQEDSDFLTESDVFTEDLIESYIQYKYDNEITPVRLRPTPQEFEMYFDC

SEQ ID NO: 2 - DNA, 1434 bp, Artificial Sequence
  KFCC10694 glnA
gtggcgtttaataccccggaagaaatagtcaagttcatcaaagacgagaacgtcgaattcgtagacgttcgcttcaccgatgtaccaggaactgaacagcacttcagcatcccagccgccctcttcgatgaagaggccatcgaagaaggcctagcattcgacggatcctcgatccgcggattcaccaccatcgatgagtctgacatgaacctcctaccagacctcggaactgccaccattgacccgttccgcaaggccaagactctgaacatcaagttcttcgttcatgatccattcacccgcgaagctttctcccgcgacccacgcaatgtggcacgcaaggcagagcagtacctcgcctccaccggcattgcagatacctgcaacttcggcgcagaagccgagttctacctctttgattcagtccgctactccaccgatattaactccagcttctaccacgttgataccaatgaaggctggtggaaccgtggccgggaaaccaaccttgatggcaccccaaaccttggcgccaagaaccgtgtcaagggcggatacttccctgttgcaccatatgaccaaaccgtggaaatccgcgatgatatggtcaactacctctcaaacgctggtttccaacttgagcgtttccaccacgaggtcggcggtggacagcaggagatcaactaccgcttcaacaccatgctgcacgcggctgatgatattcagacattcaagtacatcatcaagaacaccgctcacctccacggcaagaccgcaacctttatgcctaagccactggctggcgacaacggctctggaatgcacgcacaccagtccctatggaaggacggcaagccactcttccacgatgagtccggttacgcaggcctatctgacatcgcccgctactacattggtggcatcctgcaccacgcaggtgcagtattggcgttcaccaacccaaccctgaactcctaccaccgtttagttcctggcttcgaggcgccaatcaacttggtgtactcccagcgcaaccgctctgctgctgtacgtatcccaatcaccggatccaacccaaaggcaaagcgcatcgagttccgcgctccggacccatcaggcaacccatacttcggcttcgctgccatgatgatggctggccttgacggcatcaagaaccgcatcgagccacacgcaccagtggataaggatctctacgagcttccaccagaggaagctgcctccatcccacaggctccaacctcccttgaagcttcattgaaggctcttcaggaagattccgacttcctcaccgagtctgatgtcttcaccgaagatctcatcgagtcctacatccagtacaagtacgacaacgagatcaccccagtccgtttgcgcccaactcctcaagagttcgaaatgtacttcgactgctaa

SEQ ID NO: 3 - protein, 477 aa, Artificial Sequence
  ATCC13032 GS
VAFETPEEIVKFIKDENVEFVDVRFTDLPGTEQHFSIPAASFDADTIEEGLAFDGSSIRGFTTIDESDMNLLPDLGTATLDPFRKAKTLNVKFFVHDPFTREAFSRDPRNVARKAEQYLASTGIADTCNFGAEAEFYLFDSVRYSTEMNSGFYEVDTEEGWWNRGKETNLDGTPNLGAKNRVKGGYFPVAPYDQTVDVRDDMVRNLAASGFALERFHHEVGGGQQEINYRFNTMLHAADDIQTFKYIIKNTARLHGKAATFMPKPLAGDNGSGMHAHQSLWKDGKPLFHDESGYAGLSDIARYYIGGILHHAGAVLAFTNATLNSYHRLVPGFEAPINLVYSQRNRSAAVRIPITGSNPKAKRIEFRAPDPSGNPYLGFAAMMMAGLDGIKNRIEPHAPVDKDLYELPPEEAASIPQAPTSLEASLKALQEDTDFLTESDVFTEDLIEAYIQYKYDNEISPVRLRPTPQEFELYFDC

SEQ ID NO: 4 - DNA, 1434 bp, Artificial Sequence
  ATCC13032 glnA
gtggcgtttgaaaccccggaagaaattgtcaagttcatcaaggatgaaaacgtcgagttcgttgacgttcgattcaccgaccttcccggcaccgagcagcacttcagcatcccagctgccagcttcgatgcagatacaatcgaagaaggtctcgcattcgacggatcctcgatccgtggcttcaccacgatcgacgaatctgacatgaatctcctgccagacctcggaacggccacccttgatccattccgcaaggcaaagaccctgaacgttaagttcttcgttcacgatcctttcacccgcgaggcattctcccgcgacccacgcaacgtggcacgcaaggcagagcagtacctggcatccaccggcattgcagacacctgcaacttcggcgccgaggctgagttctacctcttcgactccgttcgctactccaccgagatgaactccggcttctacgaagtagataccgaagaaggctggtggaaccgtggcaaggaaaccaacctcgacggcaccccaaacctgggcgcaaagaaccgcgtcaagggtggctacttcccagtagcaccatacgaccaaaccgttgacgtgcgcgatgacatggttcgcaacctcgcagcttccggcttcgctcttgagcgtttccaccacgaagtcggtggcggacagcaggaaatcaactaccgcttcaacaccatgctccacgcggcagatgatatccagaccttcaagtacatcatcaagaacaccgctcgcctccacggcaaggctgcaaccttcatgcctaagccactggctggcgacaacggttccggcatgcacgctcaccagtccctctggaaggacggcaagccactcttccacgatgagtccggctacgcaggcctgtccgacatcgcccgctactacatcggcggcatcctgcaccacgcaggcgctgttctggcgttcaccaacgcaaccctgaactcctaccaccgtctggttccaggcttcgaggctccaatcaacctggtgtactcacagcgcaaccgttccgctgctgtccgtatcccaatcaccggatccaacccgaaggcaaagcgcatcgaattccgcgctccagacccatcaggcaacccatacctgggctttgcagcgatgatgatggccggcctcgacggcatcaagaaccgcatcgagccacacgctccagtggacaaggacctctacgaactaccaccagaggaagctgcatccattccacaggcaccaacctccctggaagcatccctgaaggcactgcaggaagacaccgacttcctcaccgagtctgacgtcttcaccgaggatctcatcgaggcgtacatccagtacaagtacgacaacgagatctccccagttcgcctgcgcccaaccccgcaggaattcgaattgtacttcgactgctaa

SEQ ID NO: 5 - DNA, 25 bp, Artificial Sequence
  primer 1
gggatccatacccaagatggcatgg

SEQ ID NO: 6 - DNA, 36 bp, Artificial Sequence
  primer 2
gctggaggatttagatttggtgactcctcattgaca

SEQ ID NO: 7 - DNA, 36 bp, Artificial Sequence
  primer 3
tgtcaatgaggagtcaccaaatctaaatcctccagc

SEQ ID NO: 8 - DNA, 25 bp, Artificial Sequence
  primer 4
gggatcccttaaaaagcttttcgac

SEQ ID NO: 9 - DNA, 27 bp, Artificial Sequence
  primer 5
ggaagcttcttgacctgcatgatctcg

SEQ ID NO: 10 - DNA, 36 bp, Artificial Sequence
  primer 6
gccaatcgagaacgcatgcccactactttacggtca

SEQ ID NO: 11 - DNA, 37 bp, Artificial Sequence
  primer 7
atgaccgtaaagtagtgggcatgcgttctcgattggc

SEQ ID NO: 12 - DNA, 26 bp, Artificial Sequence
  primer 8
ggaagctttacaccaaccacaactgc

SEQ ID NO: 13 - DNA, 36 bp, Artificial Sequence
  primer 9
cgaaaggattttttacccgtggcgtttgaaaccccg

SEQ ID NO: 14 - DNA, 36 bp, Artificial Sequence
  primer 10
tgccgccaggcaaattctttagcagtcgaagtacaa

SEQ ID NO: 15 - DNA, 37 bp, Artificial Sequence
  primer 11
cgaaaggattttttacccgtggcgtttaataccccgg

SEQ ID NO: 16 - DNA, 37 bp, Artificial Sequence
  primer 12
ctgccgccaggcaaattctttagcagtcgaagtacat

SEQ ID NO: 17 - DNA, 26 bp, Artificial Sequence
  primer 13
gggatccagctgccaattattccggg

SEQ ID NO: 18 - DNA, 36 bp, Artificial Sequence
  primer 14
cggggtttcaaacgccacgggtaaaaaatcctttcg

SEQ ID NO: 19 - DNA, 37 bp, Artificial Sequence
  primer 15
ccggggtattaaacgccacgggtaaaaaatcctttcg

SEQ ID NO: 20 - DNA, 36 bp, Artificial Sequence
  primer 16
ttgtacttcgactgctaaagaatttgcctggcggca

SEQ ID NO: 21 - DNA, 25 bp, Artificial Sequence
  primer 17
gggatccttcgttttatttgatgcc

SEQ ID NO: 22 - DNA, 37 bp, Artificial Sequence
  primer 18
atgtacttcgactgctaaagaatttgcctggcggcag